European Patent Application EP 4 257 605 A1, published October 11, 2023. Title: Anti-TSLP nanobodies and their applications. Applicant: SHANGHAI NOVAMAB BIOPHARMACEUTICALS CO., LTD. The sequence listing filed with the application follows.

SEQUENCE LISTING (42 sequences)

SEQ ID NO: 1 - protein, 10 aa, artificial sequence
  CDR1
GFTLDDSDMG

SEQ ID NO: 2 - protein, 7 aa, artificial sequence
  CDR2
ISSLGGT

SEQ ID NO: 3 - protein, 16 aa, artificial sequence
  CDR3
APGTDRYSDCPNEYSV

SEQ ID NO: 4 - protein, 25 aa, artificial sequence
  FR1
QVQLQESGGGSVQAGGSLRLSCTAS

SEQ ID NO: 5 - protein, 15 aa, artificial sequence
  FR2
WYRQAPGDECELVST

SEQ ID NO: 6 - protein, 38 aa, artificial sequence
  FR3
YYADSVKGRFTISHDNAKNTVYLQMNSLKPHDTAVYYC

SEQ ID NO: 7 - protein, 11 aa, artificial sequence
  FR4
WGQGTQVTVSS

SEQ ID NO: 8 - protein, 122 aa, artificial sequence
  the VHH chain of the nanobody
QVQLQESGGGSVQAGGSLRLSCTASGFTLDDSDMGWYRQAPGDECELVSTISSLGGTYYADSVKGRFTISHDNAKNTVYLQMNSLKPHDTAVYYCAPGTDRYSDCPNEYSVWGQGTQVTVSS

SEQ ID NO: 9 - DNA, 366 bp, artificial sequence
  the polynucleotide sequence
caggtgcagctgcaggagtctggaggaggctcggtgcaggctggagggtctctgagactctcctgtacagcctctggattcactttggatgattctgacatgggctggtaccgccaggctccaggggatgagtgcgagttggtctcaactattagtagtttgggtggcacatactatgcagactccgtgaagggccgattcaccatctcccatgacaacgccaagaacacggtgtatctgcaaatgaacagcctgaaacctcacgacacggccgtgtattactgtgcgccggggacagaccgttatagcgactgccctaatgagtatagcgtctggggccaggggacccaggtcaccgtctcctca

SEQ ID NO: 10 - protein, 25 aa, artificial sequence
  FR1
EVQLLESGGGLVQPGGSLRLSCTAS

SEQ ID NO: 11 - protein, 11 aa, artificial sequence
  FR4
WGQGTLVTVSS

SEQ ID NO: 12 - protein, 122 aa, artificial sequence
  the VHH chain of the nanobody
EVQLLESGGGLVQPGGSLRLSCTASGFTLDDSDMGWYRQAPGDECELVSTISSLGGTYYADSVKGRFTISHDNAKNTVYLQMNSLKPHDTAVYYCAPGTDRYSDCPNEYSVWGQGTLVTVSS

SEQ ID NO: 13 - DNA, 366 bp, artificial sequence
  the polynucleotide sequence
gaggttcaattgttggaatctggtggtggtttggttcaaccaggtggttctttgagattgtcttgtactgcttctggtttcaccttggacgattctgatatgggatggtacagacaagctccaggagatgagtgtgagttggtttctactatctcttccttgggtggaacctactacgctgattctgtcaagggtcgtttcactatttctcacgataatgctaagaacaccgtttacttgcaaatgaactctttaaagccacatgatactgccgtttactactgtgctcctggtactgatagatactctgactgtccaaacgaatactccgtttggggtcagggtactttggttactgtctcttcc

SEQ ID NO: 14 - protein, 10 aa, artificial sequence
  CDR1
GFTFDDSDMG

SEQ ID NO: 15 - protein, 7 aa, artificial sequence
  CDR2
ISSDGMT

SEQ ID NO: 16 - protein, 25 aa, artificial sequence
  CDR3
AATKYSSDYDVAEDWRRGVCGDMDY

SEQ ID NO: 17 - protein, 25 aa, artificial sequence
  FR1
QVQLQESGGGSVQAGETLRLSCTAS

SEQ ID NO: 18 - protein, 15 aa, artificial sequence
  FR2
WYRQAPGNECELVSI

SEQ ID NO: 19 - protein, 38 aa, artificial sequence
  FR3
YYADSVKGRFTISQDNAKNTVYLQMNSLKPEDTAVYYC

SEQ ID NO: 20 - protein, 11 aa, artificial sequence
  FR4
WGKGTQVTVSS

SEQ ID NO: 21 - protein, 131 aa, artificial sequence
  the VHH chain of the nanobody
QVQLQESGGGSVQAGETLRLSCTASGFTFDDSDMGWYRQAPGNECELVSIISSDGMTYYADSVKGRFTISQDNAKNTVYLQMNSLKPEDTAVYYCAATKYSSDYDVAEDWRRGVCGDMDYWGKGTQVTVSS

SEQ ID NO: 22 - DNA, 393 bp, artificial sequence
  the polynucleotide sequence
caggtgcagctgcaggagtctggaggaggctcggtgcaggctggagagactctgagactctcctgtacagcctctggattcacttttgatgattctgacatgggctggtaccgccaggctccagggaatgagtgcgagttggtctcaattattagtagtgatggtatgacatactatgcagactccgtgaagggccgattcaccatctcccaagacaacgccaagaacacggtgtatctgcaaatgaacagcctgaaacctgaggacacagccgtgtattactgtgcggcgacgaagtactccagcgactatgacgtagctgaggattggagacgcggggtctgtggagacatggactactggggcaaaggaacccaggtcaccgtctcctca

SEQ ID NO: 23 - protein, 25 aa, artificial sequence
  FR1
EVQLLESGGGLVQPGETLRLSCTAS

SEQ ID NO: 24 - protein, 11 aa, artificial sequence
  FR4
WGKGTLVTVSS

SEQ ID NO: 25 - protein, 131 aa, artificial sequence
  the VHH chain of the nanobody
EVQLLESGGGLVQPGETLRLSCTASGFTFDDSDMGWYRQAPGNECELVSIISSDGMTYYADSVKGRFTISQDNAKNTVYLQMNSLKPEDTAVYYCAATKYSSDYDVAEDWRRGVCGDMDYWGKGTLVTVSS

SEQ ID NO: 26 - DNA, 393 bp, artificial sequence
  the polynucleotide sequence
gaagtccaattgcttgaatccggtggtggattagttcaaccaggtgagaccttgagactgtcctgtaccgcttccggtttcactttcgacgactccgacatgggttggtacagacaggctccaggtaatgagtgtgagttggtttctattatttcctctgatggtatgacttactacgctgattctgttaagggtagattcactatctctcaagacaatgctaagaacactgtttacttgcaaatgaactctttgaagcctgaagataccgccgtctactactgtgctgccaccaagtactcctccgattatgatgtcgctgaagattggagaagaggagtttgtggagatatggattactggggtaaaggtactttggttaccgtttcttct

SEQ ID NO: 27 - protein, 10 aa, artificial sequence
  CDR1
GFTSGGSDMG

SEQ ID NO: 28 - protein, 7 aa, artificial sequence
  CDR2
ISSDGST

SEQ ID NO: 29 - protein, 22 aa, artificial sequence
  CDR3
AATDYGLGPPPSSTGQCYGMDY

SEQ ID NO: 30 - protein, 25 aa, artificial sequence
  FR1
QVQLQESGGGSVQAGGSLRLSCTAS

SEQ ID NO: 31 - protein, 15 aa, artificial sequence
  FR2
WYRQAPGNECDLVSY

SEQ ID NO: 32 - protein, 38 aa, artificial sequence; identical to SEQ ID NO: 19
  FR3

SEQ ID NO: 33 - protein, 11 aa, artificial sequence
  FR4
WGKGTQVTVSS

SEQ ID NO: 34 - protein, 128 aa, artificial sequence
  the VHH chain of the nanobody
QVQLQESGGGSVQAGGSLRLSCTASGFTSGGSDMGWYRQAPGNECDLVSYISSDGSTYYADSVKGRFTISQDNAKNTVYLQMNSLKPEDTAVYYCAATDYGLGPPPSSTGQCYGMDYWGKGTQVTVSS

SEQ ID NO: 35 - DNA, 384 bp, artificial sequence
  the polynucleotide sequence
caggtgcagctgcaggagtctgggggaggctcggtgcaggctggagggtctctgagactctcctgtacagcctctggattcacttctggcggttctgacatgggctggtaccgccaggctccagggaatgagtgcgacttggtctcatatattagtagtgatggtagcacatactatgcagactccgtgaagggccgattcaccatctcccaagacaacgccaagaacacggtgtatctgcaaatgaacagcctgaaacctgaggacacggccgtgtattactgtgcggccaccgactatgggttggggccgcccccttcttcgacgggccaatgttacggcatggactactggggcaaaggaacccaggtcaccgtctcctca

SEQ ID NO: 36 - protein, 25 aa, artificial sequence
  FR1
EVQLLESGGGLVQPGGSLRLSCTAS

SEQ ID NO: 37 - protein, 11 aa, artificial sequence
  FR2
WGKGTLVTVSS

SEQ ID NO: 38 - protein, 128 aa, artificial sequence
  the VHH chain of the nanobody
EVQLLESGGGLVQPGGSLRLSCTASGFTSGGSDMGWYRQAPGNECDLVSYISSDGSTYYADSVKGRFTISQDNAKNTVYLQMNSLKPEDTAVYYCAATDYGLGPPPSSTGQCYGMDYWGKGTLVTVSS

SEQ ID NO: 39 - DNA, 384 bp, artificial sequence
  the polynucleotide sequence
gaagttcagttgttggaatcaggtggtggtttggttcaaccaggaggttctctgagattgtcttgtactgcttccggtttcacttccggaggttctgacatgggatggtaccgtcaagctcctggtaacgagtgcgacttggtttcttacatctcttccgacggttccacttactacgctgattctgttaagggtagattcactatttctcaagacaacgctaagaatactgtttacttgcagatgaactctttgaagccagaggataccgctgtttactattgtgccgccactgattacggtttgggtcctccaccatcttctactggacaatgttacggtatggattactggggtaaaggtaccctggtcaccgtttcctct

SEQ ID NO: 40 - protein, 264 aa, artificial sequence
  the sequences after ligation
EVQLLESGGGLVQPGGSLRLSCTASGFTLDDSDMGWYRQAPGDECELVSTISSLGGTYYADSVKGRFTISHDNAKNTVYLQMNSLKPHDTAVYYCAPGTDRYSDCPNEYSVWGQGTLVTVSSGGGGSGGGGSGGGGSGGGGSEVQLLESGGGLVQPGGSLRLSCTASGFTLDDSDMGWYRQAPGDECELVSTISSLGGTYYADSVKGRFTISHDNAKNTVYLQMNSLKPHDTAVYYCAPGTDRYSDCPNEYSVWGQGTLVTVSS

SEQ ID NO: 41 - protein, 282 aa, artificial sequence
  the sequences after ligation
EVQLLESGGGLVQPGETLRLSCTASGFTFDDSDMGWYRQAPGNECELVSIISSDGMTYYADSVKGRFTISQDNAKNTVYLQMNSLKPEDTAVYYCAATKYSSDYDVAEDWRRGVCGDMDYWGKGTLVTVSSGGGGSGGGGSGGGGSGGGGSEVQLLESGGGLVQPGETLRLSCTASGFTFDDSDMGWYRQAPGNECELVSIISSDGMTYYADSVKGRFTISQDNAKNTVYLQMNSLKPEDTAVYYCAATKYSSDYDVAEDWRRGVCGDMDYWGKGTLVTVSS

SEQ ID NO: 42 - protein, 276 aa, artificial sequence
  the sequences after ligation
EVQLLESGGGLVQPGGSLRLSCTASGFTSGGSDMGWYRQAPGNECDLVSYISSDGSTYYADSVKGRFTISQDNAKNTVYLQMNSLKPEDTAVYYCAATDYGLGPPPSSTGQCYGMDYWGKGTLVTVSSGGGGSGGGGSGGGGSGGGGSEVQLLESGGGLVQPGGSLRLSCTASGFTSGGSDMGWYRQAPGNECDLVSYISSDGSTYYADSVKGRFTISQDNAKNTVYLQMNSLKPEDTAVYYCAATDYGLGPPPSSTGQCYGMDYWGKGTLVTVSS